European Patent Application EP 4 163 288 A1, published April 12, 2023. Title: A Novel Nucleolin-Binding Peptide and Uses Thereof. Applicant: ANYGEN CO., LTD. The sequence listing filed with the application follows.

SEQUENCE LISTING (80 sequences)

SEQ ID NO: 1 - protein, 9 aa, Artificial Sequence
  AGM-330
RHGAMVYLK

SEQ ID NO: 2 - protein, 9 aa, Artificial Sequence
  AGM-331
ADHRHRRSG

SEQ ID NO: 3 - protein, 9 aa, Artificial Sequence
  AGM-332
AVARARRRR

SEQ ID NO: 4 - protein, 9 aa, Artificial Sequence
  AGM-333
RFLKNKKAR

SEQ ID NO: 5 - protein, 9 aa, Artificial Sequence
  AGM-334
RWLKNKKAR

SEQ ID NO: 6 - protein, 9 aa, Artificial Sequence
  AGM-335
FGRLKKPLK

SEQ ID NO: 7 - protein, 9 aa, Artificial Sequence
  AGM-336
KRRRRERAG

SEQ ID NO: 8 - protein, 9 aa, Artificial Sequence
  AGM-337
KRRRKAPTD

SEQ ID NO: 9 - protein, 9 aa, Artificial Sequence
  AGM-330
KHGAMVYLK

SEQ ID NO: 10 - protein, 9 aa, Artificial Sequence
  AGM-330
RRGAMVYLK

SEQ ID NO: 11 - protein, 9 aa, Artificial Sequence
  AGM-330
RHGLMVYLK

SEQ ID NO: 12 - protein, 9 aa, Artificial Sequence
  AGM-330
RHGALVYLK

SEQ ID NO: 13 - protein, 9 aa, Artificial Sequence
  AGM-330
RHGAXVYLK

SEQ ID NO: 14 - protein, 9 aa, Artificial Sequence
  AGM-330
RHGAMAYLK

SEQ ID NO: 15 - protein, 9 aa, Artificial Sequence
  AGM-330
RHGAMVFLK

SEQ ID NO: 16 - protein, 7 aa, Artificial Sequence
  AGM-330
GAMVYLK

SEQ ID NO: 17 - protein, 11 aa, Artificial Sequence
  AGM-330
RHRHGAMVYLK

SEQ ID NO: 18 - protein, 13 aa, Artificial Sequence
  AGM-330
RHRHRHGAMVYLK

SEQ ID NO: 19 - protein, 9 aa, Artificial Sequence
  AGM-330
KLYVMAGHR

SEQ ID NO: 20 - protein, 13 aa, Artificial Sequence
  AGM-330
RHGAMVYLKLKLK

SEQ ID NO: 21 - RNA, 19 nt, Artificial Sequence
  siNCL1
gagcuaacccuuaucugua

SEQ ID NO: 22 - RNA, 19 nt, Artificial Sequence
  siNCL1
uacagauaaggguuagcuc

SEQ ID NO: 23 - RNA, 19 nt, Artificial Sequence
  siNCL2
cacaaggaaagaagacgaa

SEQ ID NO: 24 - RNA, 19 nt, Artificial Sequence
  siNCL2
uucgucuucuuuccuugug

SEQ ID NO: 25 - RNA, 19 nt, Artificial Sequence
  siNCL3
gacgaaguuugaauagcuu

SEQ ID NO: 26 - RNA, 19 nt, Artificial Sequence
  siNCL3
aagcuauucaaacuucguc

SEQ ID NO: 27 - DNA, 20 bp, Artificial Sequence
  Primer
aaagtgccccagaacccaca

SEQ ID NO: 28 - DNA, 21 bp, Artificial Sequence
  Primer
tggctgacttctcgcattagg

SEQ ID NO: 29 - DNA, 21 bp, Artificial Sequence
  Primer
gagcaatgatcttgatcttca

SEQ ID NO: 30 - DNA, 20 bp, Artificial Sequence
  Primer
agatgagtatgcctgccgtg

SEQ ID NO: 31 - protein, 11 aa, Artificial Sequence
  TAT
YGRKKRRQRRR

SEQ ID NO: 32 - protein, 13 aa, Artificial Sequence
  TAT(48-60)
GRKKRRQRRRPPQ

SEQ ID NO: 33 - protein, 9 aa, Artificial Sequence
  TAT(49-57)
RKKRRQRRR

SEQ ID NO: 34 - protein, 16 aa, Artificial Sequence
  Penetratin
RQIKIWFQNRRMKWKK

SEQ ID NO: 35 - protein, 8 aa, Artificial Sequence
  R8
RRRRRRRR

SEQ ID NO: 36 - protein, 13 aa, Artificial Sequence
  R9-TAT
GRRRRRRRRRPPQ

SEQ ID NO: 37 - protein, 21 aa, Artificial Sequence
  Pep-1
KETWWETWWTEWSQPKKKRKV

SEQ ID NO: 38 - protein, 11 aa, Artificial Sequence
  Hph-1
YARVRRRGPRR

SEQ ID NO: 39 - protein, 18 aa, Artificial Sequence
  MAP
KLALKLALKALKAALKLA

SEQ ID NO: 40 - protein, 18 aa, Artificial Sequence
  pVEC
LLIILRRRIRKQAHAHSK

SEQ ID NO: 41 - protein, 27 aa, Artificial Sequence
  MPG
GALFLGFLGAAGSTMGAWSQPKKKRKV

SEQ ID NO: 42 - protein, 27 aa, Artificial Sequence
  Transportan
GWTLNSAGYLLGKINLKALAALAKKIL

SEQ ID NO: 43 - protein, 20 aa, Artificial Sequence
  gH625
HGLASTLTRWAHYNALIRAF

SEQ ID NO: 44 - protein, 17 aa, Artificial Sequence
  VP22
NAKTRRHERRRKLAIER

SEQ ID NO: 45 - protein, 20 aa, Artificial Sequence
  DS4
VQIFRIMRILRILKLARHST

SEQ ID NO: 46 - protein, 16 aa, Artificial Sequence
  DS4-1
RIMRILRILKLARHST

SEQ ID NO: 47 - protein, 17 aa, Artificial Sequence
  DS4-2
VQIFRIMRILRILKLAR

SEQ ID NO: 48 - protein, 13 aa, Artificial Sequence
  DS4-3
RIMRILRILKLAR

SEQ ID NO: 49 - protein, 17 aa, Artificial Sequence
  KS4
FRLVRLLRFLRILLIIS

SEQ ID NO: 50 - protein, 14 aa, Artificial Sequence
  KS4-1
FRLVRLLRFLRILL

SEQ ID NO: 51 - protein, 10 aa, Artificial Sequence
  KS4-2
RLVRLLRFLR

SEQ ID NO: 52 - protein, 3 aa, Artificial Sequence
  N1
RIL

SEQ ID NO: 53 - protein, 9 aa, Artificial Sequence
  N3
RILRILRIL

SEQ ID NO: 54 - protein, 15 aa, Artificial Sequence
  N5
RILRILRILRILRIL

SEQ ID NO: 55 - protein, 21 aa, Artificial Sequence
  N7
RILRILRILRILRILRILRIL

SEQ ID NO: 56 - protein, 13 aa, Artificial Sequence
  K3
RIFWVIKLARHFI

SEQ ID NO: 57 - protein, 16 aa, Artificial Sequence
  C3
KSLRVLRVLRPLKTIK

SEQ ID NO: 58 - protein, 15 aa, Artificial Sequence
  C4
RLFRVMRLVKLLSRG

SEQ ID NO: 59 - protein, 15 aa, Artificial Sequence
  S2
RSFRLLRVFKLAKSW

SEQ ID NO: 60 - protein, 22 aa, Artificial Sequence
  S4
RVIRLARIGRILRLVKGAKGIR

SEQ ID NO: 61 - protein, 13 aa, Artificial Sequence
  D1
RAGRILRILKLAR

SEQ ID NO: 62 - protein, 13 aa, Artificial Sequence
  D2
RIMRGLRILKLAR

SEQ ID NO: 63 - protein, 13 aa, Artificial Sequence
  D3
RIMRILRLMKLAR

SEQ ID NO: 64 - protein, 13 aa, Artificial Sequence
  D4
RIMRILRILKMFR

SEQ ID NO: 65 - protein, 13 aa, Artificial Sequence
  D5
RIMRILRALKLAR

SEQ ID NO: 66 - protein, 13 aa, Artificial Sequence
  D6
RIMRGMRILKLAR

SEQ ID NO: 67 - protein, 13 aa, Artificial Sequence
  D7
RLFRILRILKLAR

SEQ ID NO: 68 - protein, 13 aa, Artificial Sequence
  D8
RIMRMVRILKLAR

SEQ ID NO: 69 - protein, 13 aa, Artificial Sequence
  D9
RIMRILRLVKLAR

SEQ ID NO: 70 - protein, 13 aa, Artificial Sequence
  D10
RIMRILRILKGVR

SEQ ID NO: 71 - protein, 13 aa, Artificial Sequence
  D11
RNLRILRILKLAR

SEQ ID NO: 72 - protein, 13 aa, Artificial Sequence
  D12
RIMRDIRILKLAR

SEQ ID NO: 73 - protein, 13 aa, Artificial Sequence
  D13
RIMRILRELKLAR

SEQ ID NO: 74 - protein, 13 aa, Artificial Sequence
  D14
RIMRILRILKQLR

SEQ ID NO: 75 - protein, 13 aa, Artificial Sequence
  D15
RIMRILRHMKLAR

SEQ ID NO: 76 - protein, 13 aa, Artificial Sequence
  D16
RIMRSVRILKLAR

SEQ ID NO: 77 - protein, 13 aa, Artificial Sequence
  D17
RTMRILRILKLAR

SEQ ID NO: 78 - protein, 13 aa, Artificial Sequence
  D18
RIMRYARILKLAR

SEQ ID NO: 79 - protein, 13 aa, Artificial Sequence
  D19
RIMRILRQIKLAR

SEQ ID NO: 80 - protein, 13 aa, Artificial Sequence
  D20
RIMRILRILKEVR